European Patent Specification EP 4 319 792 B1, published September 3, 2025. Title: RECOMBINANT LIGASE COMPOSITION AND USES THEREOF. Applicant: 10X GENOMICS, INC. The sequence listing filed with the application follows.

SEQUENCE LISTING (25 sequences)

SEQ ID NO: 1 - protein, 300 aa, Acanthocystis turfacea chlorella virus 1
MAIQKPLLAASLKKMSVDNLTFPVYATPKLDGIRALKIDGTLVSRTFKPIRNTTISKVLASLLPDGSDGEILSGKTFQDSTSTVMTTDAGIGSDTTFFWFDYVKDDPDKGYLDRIADMKTFVDQHPEILKDSCVTIVPLFPKKIDTPEELHVFEKWCLDQGFEGVMVRTAGGKYKFGRSTEKEQILVKIKQFEDDEAVVIGVSALQTNTNDKKLNQLGEMRRTSHQDGKVDLDMLGALDVDWNGIRFSIGTGFDKDTREDLWKQRDSIVGKVVKFKYFSQGIKTAPRFPVFLGFRDENDM

SEQ ID NO: 2 - DNA, 49 bp, Artificial Sequence
  source: /note="Description of Artificial Sequence: Synthetic oligonucleotide"
ctaagctctatagtcggacgtaacgagtaagaccgtcgagtcgcctagt

SEQ ID NO: 3 - DNA, 24 bp, Artificial Sequence
  source: /note="Description of Artificial Sequence: Synthetic oligonucleotide"
tactaggcgactcgacggtcttac

SEQ ID NO: 4 - DNA, 26 bp, Artificial Sequence
  source: /note="Description of Artificial Sequence: Synthetic oligonucleotide"
tcgttacgtccgactatagagcttag

SEQ ID NO: 5 - DNA, 26 bp, Artificial Sequence
  source: /note="Description of Artificial Sequence: Synthetic oligonucleotide"
tcgttacgtccgactatagagcttag

SEQ ID NO: 6 - protein, 298 aa, Artificial Sequence
  source: /note="Description of Artificial Sequence: Synthetic polypeptide"
MAITKPLLAATLENIEDVQFPCLATPKIDGIRSVKQTQMLSRTFKPIRNSVMNRLLTELLPEGSDGEISIEGATFQDTTSAVMTGHKMYNAKFSYYWFDYVTDDPLKKYIDRVEDMKNYITVHPHILEHAQVKIIPLIPVEINNITELLQYERDVLSKGFEGVMIRKPDGKYKFGRSTLKEGILLKMKQFKDAEATIISMTALFKNTNTKTKDNFGYSKRSTHKSGKVEEDVMGSIEVDYDGVVFSIGTGFDADQRRDFWQNKESYIGKMVKFKYFEMGSKDCPRFPVFIGIRHEEDR

SEQ ID NO: 7 - protein, 90 aa, Escherichia coli
MNKTQLIDVIAEKAELSKTQAKAALESTLAAITESLKEGDAVQLVGFGTFKVNHRAERTGRNPQTGKEIKIAAANVPAFVSGKALKDAVK

SEQ ID NO: 8 - DNA, 1188 bp, Artificial Sequence
  source: /note="Description of Artificial Sequence: Synthetic polynucleotide"
atggctattcagaagccgttactggcggccagcctgaagaaaatgtctgttgacaacttgactttcccggtctacgcaacgccgaaactggacggtatccgtgcgctgaagattgacggcaccctggtgtcgcgtacgttcaaaccgatccgcaatactaccatctccaaggtcctggcgagcttgctgccggacggcagcgatggtgagatcttgtctggtaagacctttcaggatagcaccagcaccgtgatgacgaccgatgcgggtatcggtagcgataccaccttcttctggtttgattacgttaaagacgacccggataagggttacctggaccgtatcgctgacatgaaaaccttcgtcgaccagcacccggaaatcctgaaagacagctgcgtgacgatcgtcccgctgttcccgaagaaaattgacacgccagaagaactgcatgtgtttgagaaatggtgtctggaccagggttttgagggcgttatggtgcgtacggccggtggcaagtataagtttggtcgcagcaccgagaaagaacaaatcctggttaagattaaacagtttgaagatgatgaagctgttgtgatcggtgtgagcgcgctgcaaaccaatacgaacgataagaaactgaatcagctgggtgagatgcgtcgtactagccaccaagacggcaaagttgacctggacatgctgggtgcgcttgacgtggactggaatggtattcgtttcagcatcggtacgggctttgataaagacacccgcgaagatctctggaaacaacgcgacagcatcgtgggtaaagtcgttaagttcaagtatttctcccagggtattaagaccgctccgcgttttcctgtgtttctgggttttcgtgacgagaacgatatgggtggcagcggtggcagcatgaataagacgcaactgattgacgtcattgcagagaaagccgagttgagcaagacccaggcgaaagccgcgctggagagcacgctggcagcgattaccgagagcctgaaagagggcgatgcagttcaactggttggcttcggcaccttcaaggtcaaccaccgtgcggagcgcaccggtcgcaacccgcagaccggtaaagaaatcaagattgcagccgcgaacgtgccggcgttcgtcagcggtaaggcactgaaagatgcagtaaag

SEQ ID NO: 9 - protein, 396 aa, Artificial Sequence
  source: /note="Description of Artificial Sequence: Synthetic polypeptide"
MAIQKPLLAASLKKMSVDNLTFPVYATPKLDGIRALKIDGTLVSRTFKPIRNTTISKVLASLLPDGSDGEILSGKTFQDSTSTVMTTDAGIGSDTTFFWFDYVKDDPDKGYLDRIADMKTFVDQHPEILKDSCVTIVPLFPKKIDTPEELHVFEKWCLDQGFEGVMVRTAGGKYKFGRSTEKEQILVKIKQFEDDEAVVIGVSALQTNTNDKKLNQLGEMRRTSHQDGKVDLDMLGALDVDWNGIRFSIGTGFDKDTREDLWKQRDSIVGKVVKFKYFSQGIKTAPRFPVFLGFRDENDMGGSGGSMNKTQLIDVIAEKAELSKTQAKAALESTLAAITESLKEGDAVQLVGFGTFKVNHRAERTGRNPQTGKEIKIAAANVPAFVSGKALKDAVK

SEQ ID NO: 10 - DNA, 5487 bp, Artificial Sequence
  source: /note="Description of Artificial Sequence: Synthetic polynucleotide"
cccgtagaaaagatcaaaggatcttcttgagatcctttttttctgcgcgtaatctgctgcttgcaaacaaaaaaaccaccgctaccagcggtggtttgtttgccggatcaagagctaccaactctttttccgaaggtaactggcttcagcagagcgcagataccaaatactgttcttctagtgtagccgtagttagcccaccacttcaagaactctgtagcaccgcctacatacctcgctctgctaatcctgttaccagtggctgctgccagtggcgataagtcgtgtcttaccgggttggactcaagacgatagttaccggataaggcgcagcggtcgggctgaacggggggttcgtgcacacagcccagcttggagcgaacgacctacaccgaactgagatacctacagcgtgagctatgagaaagcgccacgcttcccgaagggagaaaggcggacaggtatccggtaagcggcagggtcggaacaggagagcgcacgagggagcttccagggggaaacgcctggtatctttatagtcctgtcgggtttcgccacctctgacttgagcgtcgatttttgtgatgctcgtcaggggggcggagcctatggaaaaacgccagcaacgcggcctttttacggttcctggccttttgctggccttttgctcacatgttctttcctgcgttatcccctgattctgtggataaccgtattaccgcctttgagtgagctgataccgctcgccgcagccgaacgaccgagcgcagcgagtcagtgagcgaggaagcggaaggcgagagtagggaactgccaggcatcaaactaagcagaaggcccctgacggatggcctttttgcgtttctacaaactctttctgtgttgtaaaacgacggccagtcttaagctcgggccccctgggcggttctgataacgagtaatcgttaatccgcaaataacgtaaaaacccgcttcggcgggtttttttatggggggagtttagggaaagagcatttgtcagaatatttaagggcgcctgtcactttgcttgatatatgagaattatttaaccttataaatgagaaaaaagcaacgcactttaaataagatacgttgctttttcgattgatgaacacctataattaaactattcatctattatttatgattttttgtatatacaatatttctagtttgttaaagagaattaagaaaataaatctcgaaaataataaagggaaaatcagtttttgatatcaaaattatacatgtcaacgataatacaaaatataatacaaactataagatgttatcagtatttattatgcatttagaataaattttgtgtcgcccttccgcgaaattaatacgactcactataggggaattgtgagcggataacaattcccctctagaaataattttgtttaactttttgagaccttaaggaggtaaaaaatgggttctagccaccatcatcatcatcactcttccggtagcctgcaggacagcgaagtcaatcaagaggcgaagcctgaagttaagccagaagtcaaaccggaaacgcacattaacctgaaagtttcggatggctcaagcgagattttctttaagatcaagaaaaccacgccgttgcgtcgcctgatggaagcgtttgccaaacgtcagggcaaagaaatggattccctgcgcttcctgtatgacggcatccgtatccaggcagatcaagcaccggaagatctggatatggaagataacgacattattgaagcgcacagagagcaaattggtggcatggctattcagaagccgttactggcggccagcctgaagaaaatgtctgttgacaacttgactttcccggtctacgcaacgccgaaactggacggtatccgtgcgctgaagattgacggcaccctggtgtcgcgtacgttcaaaccgatccgcaatactaccatctccaaggtcctggcgagcttgctgccggacggcagcgatggtgagatcttgtctggtaagacctttcaggatagcaccagcaccgtgatgacgaccgatgcgggtatcggtagcgataccaccttcttctggtttgattacgttaaagacgacccggataagggttacctggaccgtatcgctgacatgaaaaccttcgtcgaccagcacccggaaatcctgaaagacagctgcgtgacgatcgtcccgctgttcccgaagaaaattgacacgccagaagaactgcatgtgtttgagaaatggtgtctggaccagggttttgagggcgttatggtgcgtacggccggtggcaagtataagtttggtcgcagcaccgagaaagaacaaatcctggttaagattaaacagtttgaagatgatgaagctgttgtgatcggtgtgagcgcgctgcaaaccaatacgaacgataagaaactgaatcagctgggtgagatgcgtcgtactagccaccaagacggcaaagttgacctggacatgctgggtgcgcttgacgtggactggaatggtattcgtttcagcatcggtacgggctttgataaagacacccgcgaagatctctggaaacaacgcgacagcatcgtgggtaaagtcgttaagttcaagtatttctcccagggtattaagaccgctccgcgttttcctgtgtttctgggttttcgtgacgagaacgatatgggtggcagcggtggcagcatgaataagacgcaactgattgacgtcattgcagagaaagccgagttgagcaagacccaggcgaaagccgcgctggagagcacgctggcagcgattaccgagagcctgaaagagggcgatgcagttcaactggttggcttcggcaccttcaaggtcaaccaccgtgcggagcgcaccggtcgcaacccgcagaccggtaaagaaatcaagattgcagccgcgaacgtgccggcgttcgtcagcggtaaggcactgaaagatgcagtaaagtaatgaggttgaggtctcaccccctagcataaccccttggggcctctaaacgggtcttgaggggttttttgcccctgagacgcgtcaatcgagttcgtacctaagggcgacaccccctaattagcccgggcgaaaggcccagtctttcgactgagcctttcgttttatttgatgcctggcagttccctactctcgcatggggagtccccacactaccatcggcgctacggcgtttcacttctgagttcggcatggggtcaggtgggaccaccgcgctactgccgccaggcaaacaaggggtgttatgagccatattcaggtataaatgggctcgcgataatgttcagaattggttaattggttgtaacactgacccctatttgtttatttttctaaatacattcaaatatgtatccgctcatgagacaataaccctgataaatgcttcaataatattgaaaaaggaagaatatgagccatattcaacgggaaacgtcgaggccgcgattaaattccaacatggatgctgatttatatgggtataaatgggctcgcgataatgtcgggcaatcaggtgcgacaatctatcgcttgtatgggaagcccgatgcgccagagttgtttctgaaacatggcaaaggtagcgttgccaatgatgttacagatgagatggtcagactaaactggctgacggaatttatgccacttccgaccatcaagcattttatccgtactcctgatgatgcatggttactcaccactgcgatccccggaaaaacagcgttccaggtattagaagaatatcctgattcaggtgaaaatattgttgatgcgctggcagtgttcctgcgccggttgcactcgattcctgtttgtaattgtccttttaacagcgatcgcgtatttcgcctcgctcaggcgcaatcacgaatgaataacggtttggttgatgcgagtgattttgatgacgagcgtaatggctggcctgttgaacaagtctggaaagaaatgcataaacttttgccattctcaccggattcagtcgtcactcatggtgatttctcacttgataaccttatttttgacgaggggaaattaataggttgtattgatgttggacgagtcggaatcgcagaccgataccaggatcttgccatcctatggaactgcctcggtgagttttctccttcattacagaaacggctttttcaaaaatatggtattgataatcctgatatgaataaattgcagtttcatttgatgctcgatgagtttttctaagcggcgcgccatcgaatggcgcaaaacctttcgcggtatggcatgatagcgcccggaagagagtcaattcagggtggtgaatatgaaaccagtaacgttatacgatgtcgcagagtatgccggtgtctcttatcagaccgtttcccgcgtggtgaaccaggccagccacgtttctgcgaaaacgcgggaaaaagtggaagcggcgatggcggagctgaattacattcccaaccgcgtggcacaacaactggcgggcaaacagtcgttgctgattggcgttgccacctccagtctggccctgcacgcgccgtcgcaaattgtcgcggcgattaaatctcgcgccgatcaactgggtgccagcgtggtggtgtcgatggtagaacgaagcggcgtcgaagcctgtaaagcggcggtgcacaatcttctcgcgcaacgcgtcagtgggctgatcattaactatccgctggatgaccaggatgccattgctgtggaagctgcctgcactaatgttccggcgttatttcttgatgtctctgaccagacacccatcaacagtattattttctcccatgaggacggtacgcgactgggcgtggagcatctggtcgcattgggtcaccagcaaatcgcgctgttagcgggcccattaagttctgtctcggcgcgtctgcgtctggctggctggcataaatatctcactcgcaatcaaattcagccgatagcggaacgggaaggcgactggagtgccatgtccggttttcaacaaaccatgcaaatgctgaatgagggcatcgttcccactgcgatgctggttgccaacgatcagatggcgctgggcgcaatgcgcgccattaccgagtccgggctgcgcgttggtgcggatatctcggtagtgggatacgacgataccgaagatagctcatgttatatcccgccgttaaccaccatcaaacaggattttcgcctgctggggcaaaccagcgtggaccgcttgctgcaactctctcagggccaggcggtgaagggcaatcagctgttgccagtctcactggtgaaaagaaaaaccaccctggcgcccaatacgcaaaccgcctctccccgcgcgttggccgattcattaatgcagctggcacgacaggtttcccgactggaaagcgggcagtgactcatgaccaaaatcccttaacgtgagttacgcgcgcgtcgttccactgagcgtcagac

SEQ ID NO: 11 - protein, 6 aa, Artificial Sequence
  source: /note="Description of Artificial Sequence: Synthetic peptide"
GGSGGS

SEQ ID NO: 12 - DNA, 11 bp, Artificial Sequence
  source: /note="Description of Artificial Sequence: Synthetic oligonucleotide"
aaaaaaaaaaa

SEQ ID NO: 13 - DNA, 13 bp, Artificial Sequence
  source: /note="Description of Artificial Sequence: Synthetic oligonucleotide"
ttttttttttttt

SEQ ID NO: 14 - DNA, 50 bp, Artificial Sequence
  source: /note="Description of Artificial Sequence: Synthetic oligonucleotide"
tactaggcgactcgacggtcttactcgttacgtccgactatagagcttag

SEQ ID NO: 15 - DNA, 50 bp, Artificial Sequence
  source: /note="Description of Artificial Sequence: Synthetic oligonucleotide"
tactaggcgactcgacggtcttaatcgttacgtccgactatagagcttag

SEQ ID NO: 16 - DNA, 50 bp, Artificial Sequence
  source: /note="Description of Artificial Sequence: Synthetic oligonucleotide"
tactaggcgactcgacggtcttcctcgttacgtccgactatagagcttag

SEQ ID NO: 17 - DNA, 50 bp, Artificial Sequence
  source: /note="Description of Artificial Sequence: Synthetic oligonucleotide"
tactaggcgactcgacggtctaactcgttacgtccgactatagagcttag

SEQ ID NO: 18 - DNA, 50 bp, Artificial Sequence
  source: /note="Description of Artificial Sequence: Synthetic oligonucleotide"
tactaggcgactcgacggtcttacgcgttacgtccgactatagagcttag

SEQ ID NO: 19 - DNA, 50 bp, Artificial Sequence
  source: /note="Description of Artificial Sequence: Synthetic oligonucleotide"
tactaggcgactcgacggtcttactagttacgtccgactatagagcttag

SEQ ID NO: 20 - DNA, 50 bp, Artificial Sequence
  source: /note="Description of Artificial Sequence: Synthetic oligonucleotide"
tactaggcgactcgacggtcttactccttacgtccgactatagagcttag

SEQ ID NO: 21 - DNA, 50 bp, Artificial Sequence
  source: /note="Description of Artificial Sequence: Synthetic oligonucleotide"
atgatccgctgagctgccagaatgagcaatgcaggctgatatctcgaatc

SEQ ID NO: 22 - DNA, 50 bp, Artificial Sequence; identical to SEQ ID NO: 14
  source: /note="Description of Artificial Sequence: Synthetic oligonucleotide"

SEQ ID NO: 23 - DNA, 50 bp, Artificial Sequence
  source: /note="Description of Artificial Sequence: Synthetic oligonucleotide"
tactaggcgactcgacggtcttacacgttacgtccgactatagagcttag

SEQ ID NO: 24 - DNA, 50 bp, Artificial Sequence
  source: /note="Description of Artificial Sequence: Synthetic oligonucleotide"
tactaggcgactcgacggtcttacccgttacgtccgactatagagcttag

SEQ ID NO: 25 - DNA, 50 bp, Artificial Sequence; identical to SEQ ID NO: 18
  source: /note="Description of Artificial Sequence: Synthetic oligonucleotide"